European Patent Application EP 4 162 925 A1, published April 12, 2023. Title: Composition for skin protection or wrinkle improvement including Regentide-034 and Regentide-041. Applicant: NineBiopharm Co.,Ltd. The sequence listing filed with the application follows.

SEQUENCE LISTING (4 sequences)

SEQ ID NO: 1 - protein, 10 aa, Artificial Sequence
  Peptide-034
AYGCYCGWGG

SEQ ID NO: 2 - protein, 12 aa, Artificial Sequence
  Peptide-041
CIPRGGICLVAL

SEQ ID NO: 3 - protein, 10 aa, Artificial Sequence
  Regentide-034
  NON_TER (10): amine group
AYGCYCGWGG

SEQ ID NO: 4 - protein, 12 aa, Artificial Sequence
  Regentide-041
  NON_TER (12): amine group
CIPRGGICLVAL